European Patent Application EP 4 272 822 A2, published November 8, 2023. Title: ADAMTS BINDING IMMUNOGLOBULINS. Applicant: Ablynx N.V. Application EP. The sequence listing filed with the application follows.

SEQUENCE LISTING (174 sequences)

SEQ ID NO: 1 - protein, 124 aa, synthetic construct
  REGION 1..124: note = Amino acid sequence
EVQLVESGGGLVQAGGSLRLSCAASGRTFSSYAMGWFRQAPGKERDFVAGISRSAGRTYYVDSVKGRFTISRDSAKNTVYLQMNRLKPEDTAVYYCAADLDPNRIFSRDEAAYWGQGTLVTVSS

SEQ ID NO: 2 - protein, 124 aa, synthetic construct
  REGION 1..124: note = Amino acid sequence
EVQLVESGGGLVQAGGSLRLSCAASGRTVSSYAMGWFRLAPGKEREFVAGISRSAERTYYVDSLKGRFTISRDSAKNTVYLHMNRLKPEDTAVYYCAADLDPNRIFSREEYAYWGQGTLVTVSS

SEQ ID NO: 3 - protein, 124 aa, synthetic construct
  REGION 1..124: note = Amino acid sequence
EVQLVESGGGLVQSGGSLRLSCAASGSAVSVNAMAWYRQAPGKQRDFVAGISRSAGRTYYTDSVKDRFTIARDSAKNTVYLQMNRLKPEDTAVYYCAADLDPNRIFSRDEAAYWGQGTLVTVSS

SEQ ID NO: 4 - protein, 125 aa, synthetic construct
  REGION 1..125: note = Amino acid sequence
EVQLVESGGGLVQAGDSLRLSCAASGRTFSTYFVGWFRQAPGKERDFVAAISRNGARTYYYDSVAGLFTISRDNAKNTVYLQMSSLKPEDTAVYYCAAARISPSDPSNEDGYDYWGQGTLVTVSS

SEQ ID NO: 5 - protein, 126 aa, synthetic construct
  REGION 1..126: note = Amino acid sequence
EVQLVESGGGLVQPGGSLRLSCAASRRTFSSYVMAWFRQAPGKEREFVAAISRSGDSTYYYDSLEGRFTISRDNAKNTVHLQMNSLKPEDTAVYICAASRAPSFRTIDAINYYDYWGQGTLVTVSS

SEQ ID NO: 6 - protein, 126 aa, synthetic construct
  REGION 1..126: note = Amino acid sequence
EVQLVESGGGLVQAGGSLRLSCSFSGPGRTFARYAMGWFRQAPGKNRDFITGISGSGDSTYYVYPMKDRFTISRDNAKNMVYLQMNALKPEDTAVYYCAADREINRIANDKELDFWGQGTLVTVSS

SEQ ID NO: 7 - protein, 123 aa, synthetic construct
  REGION 1..123: note = Amino acid sequence
EVQLVESGGGLVQAGGSLRLSCAASGRTTFSSYAMGWFRQAPGKERAFVATIWSGGLTVYADSAKGRFTISRDNAKNTVYLQMNSLRPEDTAVYYCAAEAVGTYYTPDGWTYWGQGTLVTVSS

SEQ ID NO: 8 - protein, 124 aa, synthetic construct
  REGION 1..124: note = Amino acid sequence
EVQLVESGGGLVQAGGSLRLSCAASGLTFRRNAMGWFRQAPGKERELLAGINWSGGTTYYVDSVKGRFTISRDNAKNTVDLQMISPKPEDTAVYYCAADGDIGTLVNDENPRYWGQGTLVTVSS

SEQ ID NO: 9 - protein, 124 aa, synthetic construct
  REGION 1..124: note = Amino acid sequence
EVQLVESGGGLVQAGGSLRLSCATSGFTFSPYYMGWFRQAPGKERDFVAAITRSRGTTYYLDSTEGRFTISRDNAKNTMYLQMNSLNPEDTAVYYCAAGRSPGDPSRTYLYEYWGQGTLVTVSS

SEQ ID NO: 10 - protein, 124 aa, synthetic construct
  REGION 1..124: note = Amino acid sequence
EVQLVESGGGLVQAGGSLRLSCAPSGFTFSPYYMGWFRQAPGKERDFVAAISRSRGTTYYLDSTEGRFTISRDNANDTVYLQMNSLNPEDTAVYYCAAGRSPGDPSRTYLYDYWGQGTLVTVSS

SEQ ID NO: 11 - protein, 124 aa, synthetic construct
  REGION 1..124: note = Amino acid sequence
EVQLVESGGGLVQAGASLRLSCATSGFTFSPYYMGWFRQAPGKERDFVAAISWSRGILYYTDSTEGRFTISRDNAKNTMYLQMDNLNPEDTAVYYCAASRSPGDPSRTYLYDYWGQGTLVTVSS

SEQ ID NO: 12 - protein, 127 aa, synthetic construct
  REGION 1..127: note = Amino acid sequence
EVQLVESGGGLVQAGGSLRLSCAASGRALSSSIMGWFRQAPGKEREFVAAITWSGGRAYYADVSDFEKGRFTISRDNGKNTVNLQMKGLKPEDTAVYYCAAALAIPVTMSPHEYPYWGQGTLVTVSS

SEQ ID NO: 13 - protein, 121 aa, synthetic construct
  REGION 1..121: note = Amino acid sequence
EVQLVESGGDLVQPGGSLRLSCAASGSDVVVNDMGWYRQAPGKQRELVADITTGGRTNYADSVKGRFTISRDNVKNTVYLQMNSLKPEDTAVYYCNAQVGDSDDDVWYAYWGQGTLVTVSS

SEQ ID NO: 14 - protein, 119 aa, synthetic construct
  REGION 1..119: note = Amino acid sequence
EVQLVESGGGLVQPGGSLRLSCAASGSIFSINVMGWYRQAPGKQRELVAAIISGGRTNYADSVKGRFTISRDNSKNTVYLQMNSLRPEDTAVYYCNAEVDAGIYAYGYWGQGTLVTVSS

SEQ ID NO: 15 - protein, 124 aa, synthetic construct
  REGION 1..124: note = Amino acid sequence
EVQLVESGGGLVQAGGSLRLSCAASGLTFSSYTMGWFRQAPGQEREFVSAISWNTFTTYYVDSVKDRFTVSRDNAKNTLYLRMNSLKPEDTAVYYCAAAGGSPRQHEPYEYRVWGQGTLVTVSS

SEQ ID NO: 16 - protein, 125 aa, synthetic construct
  REGION 1..125: note = Amino acid sequence
EVQLVESGGGFVQAGGSLRLSCVASRRTISSGTMGWFRQAPGKEREFVAAIRWSSGMPYYLDSVMDRFTISRDNAKNTVSLQMNSLQPEDTAVYYCAADRSAFRDPSFDVNYEYWGRGTLVTVSS

SEQ ID NO: 17 - protein, 125 aa, synthetic construct
  REGION 1..125: note = Amino acid sequence
EVQLVESGGGFVQAGGSLRLSCAASRRTISSGTMGWFRQAPGKEREFVAAIRWSSGITFYPDSVEGRFTISGDNAKNTVSLQMNSLKPEDTAVYYCAADRSALRDPSFEVNYEYWGRGTLVTVSS

SEQ ID NO: 18 - protein, 120 aa, synthetic construct
  REGION 1..120: note = Amino acid sequence
EVQLVESGGGLVQAGGSLRLSCVASGSIFSIDAMGWYRQAPGKERELVASVTTGASPNYGDSVTGRFTASRDRAKNALYLQMNSLKPEDTAVYYCNLIMTIPGGSQIMYWGQGTLVTVSS

SEQ ID NO: 19 - protein, 120 aa, synthetic construct
  REGION 1..120: note = Amino acid sequence
EVQLVESGGGSVQAGGSLRLSCVASGRYPMAWFRQAPGKEREFVAGVSWGGDRTYYADSVQGRFTVSRDYAKNTLYLQMNSLKPEDAAVYYCAGDPWGRLFRVKDNYSDWGQGTLVTVSS

SEQ ID NO: 20 - protein, 10 aa, synthetic construct
  REGION 1..10: note = Amino acid sequence
GRTFSSYAMG

SEQ ID NO: 21 - protein, 10 aa, synthetic construct
  REGION 1..10: note = Amino acid sequence
GRTVSSYAMG

SEQ ID NO: 22 - protein, 10 aa, synthetic construct
  REGION 1..10: note = Amino acid sequence
GSAVSVNAMA

SEQ ID NO: 23 - protein, 10 aa, synthetic construct
  REGION 1..10: note = Amino acid sequence
GRTFSTYFVG

SEQ ID NO: 24 - protein, 10 aa, synthetic construct
  REGION 1..10: note = Amino acid sequence
RRTFSSYVMA

SEQ ID NO: 25 - protein, 12 aa, synthetic construct
  REGION 1..12: note = Amino acid sequence
GPGRTFARYAMG

SEQ ID NO: 26 - protein, 11 aa, synthetic construct
  REGION 1..11: note = Amino acid sequence
GRTTFSSYAMG

SEQ ID NO: 27 - protein, 10 aa, synthetic construct
  REGION 1..10: note = Amino acid sequence
GLTFRRNAMG

SEQ ID NO: 28 - protein, 10 aa, synthetic construct
  REGION 1..10: note = Amino acid sequence
GFTFSPYYMG

SEQ ID NO: 29 - protein, 10 aa, synthetic construct
  REGION 1..10: note = Amino acid sequence
GRALSSSIMG

SEQ ID NO: 30 - protein, 10 aa, synthetic construct
  REGION 1..10: note = Amino acid sequence
GSDVVVNDMG

SEQ ID NO: 31 - protein, 10 aa, synthetic construct
  REGION 1..10: note = Amino acid sequence
GSIFSINVMG

SEQ ID NO: 32 - protein, 10 aa, synthetic construct
  REGION 1..10: note = Amino acid sequence
GLTFSSYTMG

SEQ ID NO: 33 - protein, 10 aa, synthetic construct
  REGION 1..10: note = Amino acid sequence
RRTISSGTMG

SEQ ID NO: 34 - protein, 10 aa, synthetic construct
  REGION 1..10: note = Amino acid sequence
GSIFSIDAMG

SEQ ID NO: 35 - protein, 6 aa, synthetic construct
  REGION 1..6: note = Amino acid sequence
GRYPMA

SEQ ID NO: 36 - protein, 10 aa, synthetic construct
  REGION 1..10: note = Amino acid sequence
GISRSAGRTY

SEQ ID NO: 37 - protein, 10 aa, synthetic construct
  REGION 1..10: note = Amino acid sequence
GISRSAERTY

SEQ ID NO: 38 - protein, 11 aa, synthetic construct
  REGION 1..11: note = Amino acid sequence
AISRNGARTYY

SEQ ID NO: 39 - protein, 10 aa, synthetic construct
  REGION 1..10: note = Amino acid sequence
AISRSGDSTY

SEQ ID NO: 40 - protein, 10 aa, synthetic construct
  REGION 1..10: note = Amino acid sequence
GISGSGDSTY

SEQ ID NO: 41 - protein, 9 aa, synthetic construct
  REGION 1..9: note = Amino acid sequence
TIWSGGLTV

SEQ ID NO: 42 - protein, 10 aa, synthetic construct
  REGION 1..10: note = Amino acid sequence
GINWSGGTTY

SEQ ID NO: 43 - protein, 10 aa, synthetic construct
  REGION 1..10: note = Amino acid sequence
AITRSRGTTY

SEQ ID NO: 44 - protein, 10 aa, synthetic construct
  REGION 1..10: note = Amino acid sequence
AISRSRGTTY

SEQ ID NO: 45 - protein, 10 aa, synthetic construct
  REGION 1..10: note = Amino acid sequence
AISWSRGILY

SEQ ID NO: 46 - protein, 13 aa, synthetic construct
  REGION 1..13: note = Amino acid sequence
AITWSGGRAYYAD

SEQ ID NO: 47 - protein, 9 aa, synthetic construct
  REGION 1..9: note = Amino acid sequence
DITTGGRTN

SEQ ID NO: 48 - protein, 9 aa, synthetic construct
  REGION 1..9: note = Amino acid sequence
AIISGGRTN

SEQ ID NO: 49 - protein, 10 aa, synthetic construct
  REGION 1..10: note = Amino acid sequence
AISWNTFTTY

SEQ ID NO: 50 - protein, 10 aa, synthetic construct
  REGION 1..10: note = Amino acid sequence
AIRWSSGMPY

SEQ ID NO: 51 - protein, 10 aa, synthetic construct
  REGION 1..10: note = Amino acid sequence
AIRWSSGITF

SEQ ID NO: 52 - protein, 9 aa, synthetic construct
  REGION 1..9: note = Amino acid sequence
SVTTGASPN

SEQ ID NO: 53 - protein, 10 aa, synthetic construct
  REGION 1..10: note = Amino acid sequence
GVSWGGDRTY

SEQ ID NO: 54 - protein, 15 aa, synthetic construct
  REGION 1..15: note = Amino acid sequence
DLDPNRIFSRDEAAY

SEQ ID NO: 55 - protein, 15 aa, synthetic construct
  REGION 1..15: note = Amino acid sequence
DLDPNRIFSREEYAY

SEQ ID NO: 56 - protein, 16 aa, synthetic construct
  REGION 1..16: note = Amino acid sequence
ARISPSDPSNEDGYDY

SEQ ID NO: 57 - protein, 17 aa, synthetic construct
  REGION 1..17: note = Amino acid sequence
SRAPSFRTIDAINYYDY

SEQ ID NO: 58 - protein, 15 aa, synthetic construct
  REGION 1..15: note = Amino acid sequence
DREINRIANDKELDF

SEQ ID NO: 59 - protein, 14 aa, synthetic construct
  REGION 1..14: note = Amino acid sequence
EAVGTYYTPDGWTY

SEQ ID NO: 60 - protein, 15 aa, synthetic construct
  REGION 1..15: note = Amino acid sequence
DGDIGTLVNDENPRY

SEQ ID NO: 61 - protein, 15 aa, synthetic construct
  REGION 1..15: note = Amino acid sequence
GRSPGDPSRTYLYEY

SEQ ID NO: 62 - protein, 15 aa, synthetic construct
  REGION 1..15: note = Amino acid sequence
GRSPGDPSRTYLYDY

SEQ ID NO: 63 - protein, 15 aa, synthetic construct
  REGION 1..15: note = Amino acid sequence
SRSPGDPSRTYLYDY

SEQ ID NO: 64 - protein, 15 aa, synthetic construct
  REGION 1..15: note = Amino acid sequence
ALAIPVTMSPHEYPY

SEQ ID NO: 65 - protein, 13 aa, synthetic construct
  REGION 1..13: note = Amino acid sequence
QVGDSDDDVWYAY

SEQ ID NO: 66 - protein, 11 aa, synthetic construct
  REGION 1..11: note = Amino acid sequence
EVDAGIYAYGY

SEQ ID NO: 67 - protein, 15 aa, synthetic construct
  REGION 1..15: note = Amino acid sequence
AGGSPRQHEPYEYRV

SEQ ID NO: 68 - protein, 16 aa, synthetic construct
  REGION 1..16: note = Amino acid sequence
DRSAFRDPSFDVNYEY

SEQ ID NO: 69 - protein, 16 aa, synthetic construct
  REGION 1..16: note = Amino acid sequence
DRSALRDPSFEVNYEY

SEQ ID NO: 70 - protein, 12 aa, synthetic construct
  REGION 1..12: note = Amino acid sequence
IMTIPGGSQIMY

SEQ ID NO: 71 - protein, 15 aa, synthetic construct
  REGION 1..15: note = Amino acid sequence
DPWGRLFRVKDNYSD

SEQ ID NO: 72 - protein, 25 aa, synthetic construct
  REGION 1..25: note = Amino acid sequence
EVQLVESGGGLVQAGGSLRLSCAAS

SEQ ID NO: 73 - protein, 25 aa, synthetic construct
  REGION 1..25: note = Amino acid sequence
EVQLVESGGGLVQSGGSLRLSCAAS

SEQ ID NO: 74 - protein, 25 aa, synthetic construct
  REGION 1..25: note = Amino acid sequence
EVQLVESGGGLVQAGDSLRLSCAAS

SEQ ID NO: 75 - protein, 25 aa, synthetic construct [sequence omitted]

SEQ ID NO: 76 - protein, 25 aa, synthetic construct
  REGION 1..25: note = Amino acid sequence
EVQLVESGGGLVQAGGSLRLSCSFS

SEQ ID NO: 77 - protein, 25 aa, synthetic construct
  REGION 1..25: note = Amino acid sequence
EVQLVESGGGLVQAGGSLRLSCATS

SEQ ID NO: 78 - protein, 25 aa, synthetic construct
  REGION 1..25: note = Amino acid sequence
EVQLVESGGGLVQAGGSLRLSCAPS

SEQ ID NO: 79 - protein, 25 aa, synthetic construct
  REGION 1..25: note = Amino acid sequence
EVQLVESGGGLVQAGASLRLSCATS

SEQ ID NO: 80 - protein, 25 aa, synthetic construct
  REGION 1..25: note = Amino acid sequence
EVQLVESGGDLVQPGGSLRLSCAAS

SEQ ID NO: 81 - protein, 25 aa, synthetic construct
  REGION 1..25: note = Amino acid sequence
EVQLVESGGGFVQAGGSLRLSCVAS

SEQ ID NO: 82 - protein, 25 aa, synthetic construct
  REGION 1..25: note = Amino acid sequence
EVQLVESGGGFVQAGGSLRLSCAAS

SEQ ID NO: 83 - protein, 25 aa, synthetic construct
  REGION 1..25: note = Amino acid sequence
EVQLVESGGGLVQAGGSLRLSCVAS

SEQ ID NO: 84 - protein, 25 aa, synthetic construct
  REGION 1..25: note = Amino acid sequence
EVQLVESGGGSVQAGGSLRLSCVAS

SEQ ID NO: 85 - protein, 14 aa, synthetic construct
  REGION 1..14: note = Amino acid sequence
WFRQAPGKERDFVA

SEQ ID NO: 86 - protein, 14 aa, synthetic construct
  REGION 1..14: note = Amino acid sequence
WFRLAPGKEREFVA

SEQ ID NO: 87 - protein, 14 aa, synthetic construct
  REGION 1..14: note = Amino acid sequence
WYRQAPGKQRDFVA

SEQ ID NO: 88 - protein, 14 aa, synthetic construct
  REGION 1..14: note = Amino acid sequence
WFRQAPGKEREFVA

SEQ ID NO: 89 - protein, 14 aa, synthetic construct
  REGION 1..14: note = Amino acid sequence
WFRQAPGKNRDFIT

SEQ ID NO: 90 - protein, 14 aa, synthetic construct
  REGION 1..14: note = Amino acid sequence
WFRQAPGKERAFVA

SEQ ID NO: 91 - protein, 14 aa, synthetic construct
  REGION 1..14: note = Amino acid sequence
WFRQAPGKERELLA

SEQ ID NO: 92 - protein, 14 aa, synthetic construct
  REGION 1..14: note = Amino acid sequence
WYRQAPGKQRELVA

SEQ ID NO: 93 - protein, 14 aa, synthetic construct
  REGION 1..14: note = Amino acid sequence
WFRQAPGQEREFVS

SEQ ID NO: 94 - protein, 14 aa, synthetic construct
  REGION 1..14: note = Amino acid sequence
WYRQAPGKERELVA

SEQ ID NO: 95 - protein, 39 aa, synthetic construct
  REGION 1..39: note = Amino acid sequence
YVDSVKGRFTISRDSAKNTVYLQMNRLKPEDTAVYYCAA

SEQ ID NO: 96 - protein, 39 aa, synthetic construct
  REGION 1..39: note = Amino acid sequence
YVDSLKGRFTISRDSAKNTVYLHMNRLKPEDTAVYYCAA

SEQ ID NO: 97 - protein, 39 aa, synthetic construct
  REGION 1..39: note = Amino acid sequence
YTDSVKDRFTIARDSAKNTVYLQMNRLKPEDTAVYYCAA

SEQ ID NO: 98 - protein, 38 aa, synthetic construct
  REGION 1..38: note = Amino acid sequence
YDSVAGLFTISRDNAKNTVYLQMSSLKPEDTAVYYCAA

SEQ ID NO: 99 - protein, 39 aa, synthetic construct
  REGION 1..39: note = Amino acid sequence
YYDSLEGRFTISRDNAKNTVHLQMNSLKPEDTAVYICAA

SEQ ID NO: 100 - protein, 39 aa, synthetic construct
  REGION 1..39: note = Amino acid sequence
YVYPMKDRFTISRDNAKNMVYLQMNALKPEDTAVYYCAA

SEQ ID NO: 101 - protein, 39 aa, synthetic construct
  REGION 1..39: note = Amino acid sequence
YADSAKGRFTISRDNAKNTVYLQMNSLRPEDTAVYYCAA

SEQ ID NO: 102 - protein, 39 aa, synthetic construct
  REGION 1..39: note = Amino acid sequence
YVDSVKGRFTISRDNAKNTVDLQMISPKPEDTAVYYCAA

SEQ ID NO: 103 - protein, 39 aa, synthetic construct
  REGION 1..39: note = Amino acid sequence
YLDSTEGRFTISRDNAKNTMYLQMNSLNPEDTAVYYCAA

SEQ ID NO: 104 - protein, 39 aa, synthetic construct
  REGION 1..39: note = Amino acid sequence
YLDSTEGRFTISRDNANDTVYLQMNSLNPEDTAVYYCAA

SEQ ID NO: 105 - protein, 39 aa, synthetic construct
  REGION 1..39: note = Amino acid sequence
YTDSTEGRFTISRDNAKNTMYLQMDNLNPEDTAVYYCAA

SEQ ID NO: 106 - protein, 39 aa, synthetic construct
  REGION 1..39: note = Amino acid sequence
VSDFEKGRFTISRDNGKNTVNLQMKGLKPEDTAVYYCAA

SEQ ID NO: 107 - protein, 39 aa, synthetic construct
  REGION 1..39: note = Amino acid sequence
YADSVKGRFTISRDNVKNTVYLQMNSLKPEDTAVYYCNA

SEQ ID NO: 108 - protein, 39 aa, synthetic construct
  REGION 1..39: note = Amino acid sequence
YADSVKGRFTISRDNSKNTVYLQMNSLRPEDTAVYYCNA

SEQ ID NO: 109 - protein, 39 aa, synthetic construct
  REGION 1..39: note = Amino acid sequence
YVDSVKDRFTVSRDNAKNTLYLRMNSLKPEDTAVYYCAA

SEQ ID NO: 110 - protein, 39 aa, synthetic construct
  REGION 1..39: note = Amino acid sequence
YLDSVMDRFTISRDNAKNTVSLQMNSLQPEDTAVYYCAA

SEQ ID NO: 111 - protein, 39 aa, synthetic construct
  REGION 1..39: note = Amino acid sequence
YPDSVEGRFTISGDNAKNTVSLQMNSLKPEDTAVYYCAA

SEQ ID NO: 112 - protein, 39 aa, synthetic construct
  REGION 1..39: note = Amino acid sequence
YGDSVTGRFTASRDRAKNALYLQMNSLKPEDTAVYYCNL

SEQ ID NO: 113 - protein, 39 aa, synthetic construct
  REGION 1..39: note = Amino acid sequence
YADSVQGRFTVSRDYAKNTLYLQMNSLKPEDAAVYYCAG

SEQ ID NO: 114 - protein, 11 aa, synthetic construct
  REGION 1..11: note = Amino acid sequence
WGQGTLVTVSS

SEQ ID NO: 115 - protein, 11 aa, synthetic construct
  REGION 1..11: note = Amino acid sequence
WGRGTLVTVSS

SEQ ID NO: 116 - protein, 120 aa, synthetic construct
  REGION 1..120: note = Amino acid sequence
EVQLVESGGGSVQAGGSLRLSCVASGRYPMAWFRQAPGKEREFVAGVSWGGDRTYYADSVQGRFTVSRDYAKNTLYLQMNSLKPEDAAVYYCAGDPWGRLFRVKDQYSDWGQGTLVTVSS

SEQ ID NO: 117 - protein, 124 aa, synthetic construct
  REGION 1..124: note = Amino acid sequence
EVQLVESGGGLVQAGGSLRLSCAASGLTFRRNAMGWFRQAPGKERELLAGISWSGGTTYYVDSVKGRFTISRDNAKNTVDLQMISPKPEDTAVYYCAADGDIGTLVNDENPRYWGQGTLVTVSS

SEQ ID NO: 118 - protein, 15 aa, synthetic construct
  REGION 1..15: note = Amino acid sequence
DPWGRLFRVKDQYSD

SEQ ID NO: 119 - protein, 10 aa, synthetic construct
  REGION 1..10: note = Amino acid sequence
GISWSGGTTY

SEQ ID NO: 120 - protein, 274 aa, synthetic construct
  REGION 1..274: note = Amino acid sequence
EVQLVESGGGLVQAGGSLRLSCAASGRTFSSYAMGWFRQAPGKERDFVAGISRSAGRTYYVDSVKGRFTISRDSAKNTVYLQMNRLKPEDTAVYYCAADLDPNRIFSRDEAAYWGQGTLVTVSSGGGGSGGGGSGGGGSGGGGSGGGGSGGGGSGGGGSEVQLVESGGGLVQPGNSLRLSCAASGFTFSSFGMSWVRQAPGKGLEWVSSISGSGSDTLYADSVKGRFTISRDNAKTTLYLQMNSLRPEDTAVYYCTIGGSLSRSSQGTLVTVSS

SEQ ID NO: 121 - protein, 276 aa, synthetic construct
  REGION 1..276: note = Amino acid sequence
EVQLVESGGGLVQAGGSLRLSCSFSGPGRTFARYAMGWFRQAPGKNRDFITGISGSGDSTYYVYPMKDRFTISRDNAKNMVYLQMNALKPEDTAVYYCAADREINRIANDKELDFWGQGTLVTVSSGGGGSGGGGSGGGGSGGGGSGGGGSGGGGSGGGGSEVQLVESGGGLVQPGNSLRLSCAASGFTFSSFGMSWVRQAPGKGLEWVSSISGSGSDTLYADSVKGRFTISRDNAKTTLYLQMNSLRPEDTAVYYCTIGGSLSRSSQGTLVTVSS

SEQ ID NO: 122 - protein, 274 aa, synthetic construct
  REGION 1..274: note = Amino acid sequence
EVQLVESGGGLVQAGGSLRLSCAASGRTVSSYAMGWFRLAPGKEREFVAGISRSAERTYYVDSLKGRFTISRDSAKNTVYLHMNRLKPEDTAVYYCAADLDPNRIFSREEYAYWGQGTLVTVSSGGGGSGGGGSGGGGSGGGGSGGGGSGGGGSGGGGSEVQLVESGGGLVQPGNSLRLSCAASGFTFSSFGMSWVRQAPGKGLEWVSSISGSGSDTLYADSVKGRFTISRDNAKTTLYLQMNSLRPEDTAVYYCTIGGSLSRSSQGTLVTVSS

SEQ ID NO: 123 - protein, 274 aa, synthetic construct
  REGION 1..274: note = Amino acid sequence
EVQLVESGGGLVQAGGSLRLSCAASGLTFRRNAMGWFRQAPGKERELLAGISWSGGTTYYVDSVKGRFTISRDNAKNTVDLQMISPKPEDTAVYYCAADGDIGTLVNDENPRYWGQGTLVTVSSGGGGSGGGGSGGGGSGGGGSGGGGSGGGGSGGGGSEVQLVESGGGLVQPGNSLRLSCAASGFTFSSFGMSWVRQAPGKGLEWVSSISGSGSDTLYADSVKGRFTISRDNAKTTLYLQMNSLRPEDTAVYYCTIGGSLSRSSQGTLVTVSS

SEQ ID NO: 124 - protein, 274 aa, synthetic construct
  REGION 1..274: note = Amino acid sequence
EVQLVESGGGLVQSGGSLRLSCAASGSAVSVNAMAWYRQAPGKQRDFVAGISRSAGRTYYTDSVKDRFTIARDSAKNTVYLQMNRLKPEDTAVYYCAADLDPNRIFSRDEAAYWGQGTLVTVSSGGGGSGGGGSGGGGSGGGGSGGGGSGGGGSGGGGSEVQLVESGGGLVQPGNSLRLSCAASGFTFSSFGMSWVRQAPGKGLEWVSSISGSGSDTLYADSVKGRFTISRDNAKTTLYLQMNSLRPEDTAVYYCTIGGSLSRSSQGTLVTVSS

SEQ ID NO: 125 - protein, 275 aa, synthetic construct
  REGION 1..275: note = Amino acid sequence
EVQLVESGGGFVQAGGSLRLSCVASRRTISSGTMGWFRQAPGKEREFVAAIRWSSGMPYYLDSVMDRFTISRDNAKNTVSLQMNSLQPEDTAVYYCAADRSAFRDPSFDVNYEYWGRGTLVTVSSGGGGSGGGGSGGGGSGGGGSGGGGSGGGGSGGGGSEVQLVESGGGLVQPGNSLRLSCAASGFTFSSFGMSWVRQAPGKGLEWVSSISGSGSDTLYADSVKGRFTISRDNAKTTLYLQMNSLRPEDTAVYYCTIGGSLSRSSQGTLVTVSS

SEQ ID NO: 126 - protein, 429 aa, synthetic construct
  REGION 1..429: note = Amino acid sequence
EVQLVESGGGLVQAGGSLRLSCAASGRTVSSYAMGWFRLAPGKEREFVAGISRSAERTYYVDSLKGRFTISRDSAKNTVYLHMNRLKPEDTAVYYCAADLDPNRIFSREEYAYWGQGTLVTVSSGGGGSGGGGSGGGGSGGGGSGGGGSGGGGSGGGGSEVQLVESGGGSVQAGGSLRLSCVASGRYPMAWFRQAPGKEREFVAGVSWGGDRTYYADSVQGRFTVSRDYAKNTLYLQMNSLKPEDAAVYYCAGDPWGRLFRVKDQYSDWGQGTLVTVSSGGGGSGGGGSGGGGSGGGGSGGGGSGGGGSGGGGSEVQLVESGGGLVQPGNSLRLSCAASGFTFSSFGMSWVRQAPGKGLEWVSSISGSGSDTLYADSVKGRFTISRDNAKTTLYLQMNSLRPEDTAVYYCTIGGSLSRSSQGTLVTVSS

SEQ ID NO: 127 - protein, 429 aa, synthetic construct
  REGION 1..429: note = Amino acid sequence
EVQLVESGGGLVQAGGSLRLSCAASGLTFRRNAMGWFRQAPGKERELLAGISWSGGTTYYVDSVKGRFTISRDNAKNTVDLQMISPKPEDTAVYYCAADGDIGTLVNDENPRYWGQGTLVTVSSGGGGSGGGGSGGGGSGGGGSGGGGSGGGGSGGGGSEVQLVESGGGSVQAGGSLRLSCVASGRYPMAWFRQAPGKEREFVAGVSWGGDRTYYADSVQGRFTVSRDYAKNTLYLQMNSLKPEDAAVYYCAGDPWGRLFRVKDQYSDWGQGTLVTVSSGGGGSGGGGSGGGGSGGGGSGGGGSGGGGSGGGGSEVQLVESGGGLVQPGNSLRLSCAASGFTFSSFGMSWVRQAPGKGLEWVSSISGSGSDTLYADSVKGRFTISRDNAKTTLYLQMNSLRPEDTAVYYCTIGGSLSRSSQGTLVTVSS

SEQ ID NO: 128 - protein, 429 aa, synthetic construct
  REGION 1..429: note = Amino acid sequence
EVQLVESGGGLVQSGGSLRLSCAASGSAVSVNAMAWYRQAPGKQRDFVAGISRSAGRTYYTDSVKDRFTIARDSAKNTVYLQMNRLKPEDTAVYYCAADLDPNRIFSRDEAAYWGQGTLVTVSSGGGGSGGGGSGGGGSGGGGSGGGGSGGGGSGGGGSEVQLVESGGGSVQAGGSLRLSCVASGRYPMAWFRQAPGKEREFVAGVSWGGDRTYYADSVQGRFTVSRDYAKNTLYLQMNSLKPEDAAVYYCAGDPWGRLFRVKDQYSDWGQGTLVTVSSGGGGSGGGGSGGGGSGGGGSGGGGSGGGGSGGGGSEVQLVESGGGLVQPGNSLRLSCAASGFTFSSFGMSWVRQAPGKGLEWVSSISGSGSDTLYADSVKGRFTISRDNAKTTLYLQMNSLRPEDTAVYYCTIGGSLSRSSQGTLVTVSS

SEQ ID NO: 129 - protein, 275 aa, synthetic construct
  REGION 1..275: note = Amino acid sequence
DVQLVESGGGVVQPGGSLRLSCAASGRTVSSYAMGWFRQAPGKEREFVAGISRSAERTYYVDSLKGRFTISRDNSKNTVYLQMNSLRPEDTALYYCAADLDPNRIFSREEYAYWGQGTLVTVSSGGGGSGGGGSGGGGSGGGGSGGGGSGGGGSGGGGSEVQLVESGGGVVQPGNSLRLSCAASGFTFSSFGMSWVRQAPGKGLEWVSSISGSGSDTLYADSVKGRFTISRDNAKTTLYLQMNSLRPEDTALYYCTIGGSLSRSSQGTLVTVSSA

SEQ ID NO: 130 - protein, 430 aa, synthetic construct
  REGION 1..430: note = Amino acid sequence
DVQLVESGGGVVQPGGSLRLSCAASGRTVSSYAMGWFRQAPGKEREFVAGISRSAERTYYVDSLKGRFTISRDNSKNTVYLQMNSLRPEDTALYYCAADLDPNRIFSREEYAYWGQGTLVTVSSGGGGSGGGGSGGGGSGGGGSGGGGSGGGGSGGGGSEVQLVESGGGVVQPGGSLRLSCAASGRYPMAWFRQAPGKEREFVAGVSWGGDRTYYADSVKGRFTISRDYSKNTLYLQMNSLRPEDTALYYCAGDPFGRLFRVKDQYSDWGQGTLVTVSSGGGGSGGGGSGGGGSGGGGSGGGGSGGGGSGGGGSEVQLVESGGGVVQPGNSLRLSCAASGFTFSSFGMSWVRQAPGKGLEWVSSISGSGSDTLYADSVKGRFTISRDNAKTTLYLQMNSLRPEDTALYYCTIGGSLSRSSQGTLVTVSSA

SEQ ID NO: 131 - protein, 115 aa, synthetic construct [sequence omitted]

SEQ ID NO: 132 - protein, 115 aa, synthetic construct [sequence omitted]

SEQ ID NO: 133 - protein, 116 aa, synthetic construct
  REGION 1..116: note = Amino acid sequence
EVQLVESGGGVVQPGNSLRLSCAASGFTFSSFGMSWVRQAPGKGLEWVSSISGSGSDTLYADSVKGRFTISRDNAKTTLYLQMNSLRPEDTATYYCTIGGSLSRSSQGTLVTVSSA

SEQ ID NO: 134 - protein, 116 aa, synthetic construct
  REGION 1..116: note = Amino acid sequence
EVQLVESGGGVVQPGGSLRLSCAASGFTFRSFGMSWVRQAPGKGPEWVSSISGSGSDTLYADSVKGRFTISRDNSKNTLYLQMNSLRPEDTATYYCTIGGSLSRSSQGTLVTVSSA

SEQ ID NO: 135 - protein, 115 aa, synthetic construct [sequence omitted]

SEQ ID NO: 136 - protein, 116 aa, synthetic construct
  REGION 1..116: note = Amino acid sequence
EVQLVESGGGLVQPGNSLRLSCAASGFTFSSFGMSWVRQAPGKGLEWVSSISGSGSDTLYADSVKGRFTISRDNAKTTLYLQMNSLRPEDTAVYYCTIGGSLSRSSQGTLVKVSSA

SEQ ID NO: 137 - protein, 115 aa, synthetic construct
  REGION 1..115: note = Amino acid sequence
EVQLVESGGGVVQPGNSLRLSCAASGFTFSSFGMSWVRQAPGKGLEWVSSISGSGSDTLYADSVKGRFTISRDNAKTTLYLQMNSLRPEDTALYYCTIGGSLSRSSQGTLVTVSS

SEQ ID NO: 138 - protein, 116 aa, synthetic construct
  REGION 1..116: note = Amino acid sequence
EVQLVESGGGVVQPGNSLRLSCAASGFTFSSFGMSWVRQAPGKGLEWVSSISGSGSDTLYADSVKGRFTISRDNAKTTLYLQMNSLRPEDTALYYCTIGGSLSRSSQGTLVTVSSA

SEQ ID NO: 139 - protein, 117 aa, synthetic construct
  REGION 1..117: note = Amino acid sequence
EVQLVESGGGVVQPGNSLRLSCAASGFTFSSFGMSWVRQAPGKGLEWVSSISGSGSDTLYADSVKGRFTISRDNAKTTLYLQMNSLRPEDTALYYCTIGGSLSRSSQGTLVTVSSAA

SEQ ID NO: 140 - protein, 118 aa, synthetic construct
  REGION 1..118: note = Amino acid sequence
EVQLVESGGGVVQPGNSLRLSCAASGFTFSSFGMSWVRQAPGKGLEWVSSISGSGSDTLYADSVKGRFTISRDNAKTTLYLQMNSLRPEDTALYYCTIGGSLSRSSQGTLVTVSSAAA

SEQ ID NO: 141 - protein, 116 aa, synthetic construct
  REGION 1..116: note = Amino acid sequence
EVQLVESGGGVVQPGNSLRLSCAASGFTFSSFGMSWVRQAPGKGLEWVSSISGSGSDTLYADSVKGRFTISRDNAKTTLYLQMNSLRPEDTALYYCTIGGSLSRSSQGTLVTVSSG

SEQ ID NO: 142 - protein, 117 aa, synthetic construct
  REGION 1..117: note = Amino acid sequence
EVQLVESGGGVVQPGNSLRLSCAASGFTFSSFGMSWVRQAPGKGLEWVSSISGSGSDTLYADSVKGRFTISRDNAKTTLYLQMNSLRPEDTALYYCTIGGSLSRSSQGTLVTVSSGG

SEQ ID NO: 143 - protein, 118 aa, synthetic construct
  REGION 1..118: note = Amino acid sequence
EVQLVESGGGVVQPGNSLRLSCAASGFTFSSFGMSWVRQAPGKGLEWVSSISGSGSDTLYADSVKGRFTISRDNAKTTLYLQMNSLRPEDTALYYCTIGGSLSRSSQGTLVTVSSGGG

SEQ ID NO: 144 - protein, 115 aa, synthetic construct
  REGION 1..115: note = Amino acid sequence
EVQLVESGGGVVQPGGSLRLSCAASGFTFRSFGMSWVRQAPGKGPEWVSSISGSGSDTLYADSVKGRFTISRDNSKNTLYLQMNSLRPEDTALYYCTIGGSLSRSSQGTLVTVSS

SEQ ID NO: 145 - protein, 116 aa, synthetic construct
  REGION 1..116: note = Amino acid sequence
EVQLVESGGGVVQPGGSLRLSCAASGFTFRSFGMSWVRQAPGKGPEWVSSISGSGSDTLYADSVKGRFTISRDNSKNTLYLQMNSLRPEDTALYYCTIGGSLSRSSQGTLVTVSSA

SEQ ID NO: 146 - protein, 5 aa, synthetic construct
  REGION 1..5: note = Amino acid sequence
SFGMS

SEQ ID NO: 147 - protein, 17 aa, synthetic construct
  REGION 1..17: note = Amino acid sequence
SISGSGSDTLYADSVKG

SEQ ID NO: 148 - protein, 6 aa, synthetic construct
  REGION 1..6: note = Amino acid sequence
GGSLSR

SEQ ID NO: 149 - protein, 930 aa, Homo sapiens
  REGION 1..930: note = Amino acid sequence
MLLGWASLLLCAFRLPLAAVGPAATPAQDKAGQPPTAAAAAQPRRRQGEEVQERAEPPGHPHPLAQRRRSKGLVQNIDQLYSGGGKVGYLVYAGGRRFLLDLERDGSVGIAGFVPAGGGTSAPWRHRSHCFYRGTVDGSPRSLAVFDLCGGLDGFFAVKHARYTLKPLLRGPWAEEEKGRVYGDGSARILHVYTREGFSFEALPPRASCETPASTPEAHEHAPAHSNPSGRAALASQLLDQSALSPAGGSGPQTWWRRRRRSISRARQVELLLVADASMARLYGRGLQHYLLTLASIANRLYSHASIENHIRLAVVKVVVLGDKDKSLEVSKNAATTLKNFCKWQHQHNQLGDDHEEHYDAAILFTREDLCGHHSCDTLGMADVGTICSPERSCAVIEDDGLHAAFTVAHEIGHLLGLSHDDSKFCEETFGSTEDKRLMSSILTSIDASKPWSKCTSATITEFLDDGHGNCLLDLPRKQILGPEELPGQTYDATQQCNLTFGPEYSVCPGMDVCARLWCAVVRQGQMVCLTKKLPAVEGTPCGKGRICLQGKCVDKTKKKYYSTSSHGNWGSWGSWGQCSRSCGGGVQFAYRHCNNPAPRNNGRYCTGKRAIYRSCSLMPCPPNGKSFRHEQCEAKNGYQSDAKGVKTFVEWVPKYAGVLPADVCKLTCRAKGTGYYVVFSPKVTDGTECRLYSNSVCVRGKCVRTGCDGIIGSKLQYDKCGVCGGDNSSCTKIVGTFNKKSKGYTDVVRIPEGATHIKVRQFKAKDQTRFTAYLALKKKNGEYLINGKYMISTSETIIDINGTVMNYSGWSHRDDFLHGMGYSATKEILIVQILATDPTKPLDVRYSFFVPKKSTPKVNSVTSHGSNKVGSHTSQPQWVTGPWLACSRTCDTGWHTRTVQCQDGNRKLAKGCPLSQRPSAFKQCLLKKC

SEQ ID NO: 150 - protein, 636 aa, synthetic construct
  REGION 1..636: note = Amino acid sequence
MLLGWAALMLCALRLPPVAAGPTAAPAQDKAGQPRAAAVAAAAQPRGRRGEEAQEPAEPPGHPHPLAPQRGSRGLVQNIDQLYSGGGKVGYLVYAGGRRFLLDLERDDSVGAAGLVPAGGGPNATRRHRGHCFYRGTVDGSPRSLAVFDLCGGLDGFFAVKRARYTLQPLLRGPWAEAEGDARVYGDESARILHVYTREGFSFEALPPRTSCETHASPPGARERPPAPSRPDGRWALAPQQLPGQSAPSSDGSQGPRTWWRRRRRSISRARQVELLLVADASMARMYGRGLQHYLLTLASIANKLYSHASIENHIRLVVVKVVVLGDKDKSLEVSKNAATTLKNFCKWQHQHNQLGDDHEEHYDAAILFTREDLCGHHSCDTLGMADVGTICSPERSCAVIEDDGLHAAFTVAHEIGHLLGLSHDDSKFCEENFGSTEDKRLMSSILTSIDASKPWSKCTSATITEFLDDGHGNCLLDLPRKQIPGPEELPGQTYDASQQCNLTFGPEYSVCPGMDVCARLWCAVVRQGQMVCLTKKLPAVEGTPCGKGRICLQGKCVDKTKKKYYSTSSHGNWGSWGSWGQCSRSCGGGVQFAYRHCNNPAPRNNGRYCTGKRAIYRSCSVTPCPHHHHHHHHHH

SEQ ID NO: 151 - protein, 629 aa, synthetic construct
  REGION 1..629: note = Amino acid sequence
MRLEWASLLLLLLLLCASCLALAADNPAAAPAQDKTRQPRAAAAAAQPDQRQWEETQERGHPQPLARQRRSSGLVQNIDQLYSGGGKVGYLVYAGGRRFLLDLERDDTVGAAGGIVTAGGLSASSGHRGHCFYRGTVDGSPRSLAVFDLCGGLDGFFAVKHARYTLKPLLRGSWAESERVYGDGSSRILHVYTREGFSFEALPPRTSCETPASPSGAQESPSVHSSSRRRTELAPQLLDHSAFSPAGNAGPQTWWRRRRRSISRARQVELLLVADSSMAKMYGRGLQHYLLTLASIANRLYSHASIENHIRLAVVKVVVLTDKSLEVSKNAATTLKNFCKWQHQHNQLGDDHEEHYDAAILFTREDLCGHHSCDTLGMADVGTICSPERSCAVIEDDGLHAAFTVAHEIGHLLGLSHDDSKFCEENFGSTEDKRLMSSILTSIDASKPWSKCTSATITEFLDDGHGNCLLDVPRKQILGPEELPGQTYDATQQCNLTFGPEYSVCPGMDVCARLWCAVVRQGQMVCLTKKLPAVEGTPCGKGRICLQGKCVDKTKKKYYSTSSHGNWGSWGPWGQCSRSCGGGVQFAYRHCNNPAPRNSGRYCTGKRAIYRSCSVIPCPHHHHHHHHHH

SEQ ID NO: 152 - protein, 632 aa, synthetic construct
  REGION 1..632: note = Amino acid sequence
MLLGWASLLLCAFRLPQAAASAAAAPAQDKAGQPRAAAAAPQPRRRQGEHAPLRVEPPGHPHALAPQRRGRGLLQSIDRLYSGGGKVGYLVYAGGRRFLLDLERDGSVGAAGLFPAGGGLSAPRRHRSHCFYRGTVDGSPRSLAVFDLCGGLRGFFAVKHARYTVKPLLRGPWAEADTPRVYGDESARIPHVYTREGFSFEALPPRASCETPASQPGPHERPPAHNSPGRHSTVDPQLPELSALSPAGDPGQQIWWRRRRRSISRARQVELLLVADGSMAKMYGRGLQHYLLTLASIANRLYSHASIENHIRLAVVKVVVLGDKDKSLEVSKNAATTLKNFCKWQHQHNQLGDDHEEHYDAAILFTREDLCGHHSCDTLGMADVGTICSPERSCAVIEDDGLHAAFTVAHEIGHLLGLSHDDSKFCEENFGLTEDKRLMSSILTSIDASKPWSKCTSATMTEFLDDGHGNCLLDVPRKQIPSPEELPGQTYDATQQCNLTFGPEYSVCPGMDVCARLWCAVVRQGQMVCLTKKLPAVEGTPCGKGRICLQGKCVDKTKKKYYSTSSHGNWGSWGPWGQCSRSCGGGVQFAYRHCNNPAPRNSGRYCTGKRAIYRSCSVTPCPHHHHHHHHHH

SEQ ID NO: 153 - protein, 632 aa, synthetic construct
  REGION 1..632: note = Amino acid sequence
MRLEWAPLLLLLLLLSASCLSLAADSPAAAPAQDKTRQPQAAAAAAEPDQPQGEETRERGHLQPLAGQRRSGGLVQNIDQLYSGGGKVGYLVYAGGRRFLLDLERDDTVGAAGSIVTAGGGLSASSGHRGHCFYRGTVDGSPRSLAVFDLCGGLDGFFAVKHARYTLKPLLRGSWAEYERIYGDGSSRILHVYNREGFSFEALPPRASCETPASPSGPQESPSVHSRSRRRSALAPQLLDHSAFSPSGNAGPQTWWRRRRRSISRARQVELLLVADSSMARMYGRGLQHYLLTLASIANRLYSHASIENHIRLAVVKVVVLTDKDTSLEVSKNAATTLKNFCKWQHQHNQLGDDHEEHYDAAILFTREDLCGHHSCDTLGMADVGTICSPERSCAVIEDDGLHAAFTVAHEIGHLLGLSHDDSKFCEENFGTTEDKRLMSSILTSIDASKPWSKCTSATITEFLDDGHGNCLLDLPRKQILGPEELPGQTYDATQQCNLTFGPEYSVCPGMDVCARLWCAVVRQGQMVCLTKKLPAVEGTPCGKGRVCLQGKCVDKTKKKYYSTSSHGNWGSWGPWGQCSRSCGGGVQFAYRHCNNPAPRNSGRYCTGKRAIYRSCSVTPCPHHHHHHHHHH

SEQ ID NO: 154 - protein, 632 aa, synthetic construct
  REGION 1..632: note = Amino acid sequence
MLLGWASLLLCAFRLPLAAAGPAAAPAQDKAGQPATAAAAAQPRRRQGEEVQERTEPPGHPHPLAQRRSSKGLVQNIDQLYSGGGKVGYLVYAGGRRFLLDLERDGSVGTAGFVPTEGGTSAPWRHRSHCFYRGTVDGSPRSLAVFDLCGGLDGFFAVKHARYTLKPLLRGPWAEEETRRVYGDGSARILHVYTREGFSFEALQPRASCETPASTPEPHERPPAHSNPGGRAALASQLLDQSAVSPAGGPGPQTWWRRRRRSISRARQVELLLVADASMARLYGRGLQHYLLTLASIANRLYSHASIENHIRLAVVKVVVLGDKDKSLEVSKNAATTLKNFCKWQHQHNQLGDDHEEHYDAAILFTREDLCGHHSCDTLGMADVGTICSPERSCAVIEDDGLHAAFTVAHEIGHLLGLSHDDSKFCEETFGSTEDKRLMSSILTSIDASKPWSKCTSATITEFLDDGHGNCLLDQPRKQILGPEELPGQTYDATQQCNLTFGPEYSVCPGMDVCARLWCAVVRQGQMVCLTKKLPAVEGTPCGKGRICLQGKCVDKTKKKYYSTSSHGNWGSWGSWGQCSRSCGGGVQFAYRHCNNPAPRNNGRYCTGKRAIYRSCGLMPCPHHHHHHHHHH

SEQ ID NO: 155 - protein, 2415 aa, synthetic construct
  REGION 1..2415: note = Amino acid sequence
MTTLLWVFVTLRVITAAVTVETSDHDNSLSVSIPQPSPLRVLLGTSLTIPCYFIDPMHPVTTAPSTAPLAPRIKWSRVSKEKEVVLLVATEGRVRVNSAYQDKVSLPNYPAIPSDATLEVQSLRSNDSGVYRCEVMHGIEDSEATLEVVVKGIVFHYRAISTRYTLDFDRAQRACLQNSAIIATPEQLQAAYEDGFHQCDAGWLADQTVRYPIHTPREGCYGDKDEFPGVRTYGIRDTNETYDVYCFAEEMEGEVFYATSPEKFTFQEAANECRRLGARLATTGHVYLAWQAGMDMCSAGWLADRSVRYPISKARPNCGGNLLGVRTVYVHANQTGYPDPSSRYDAICYTGEDFVDIPENFFGVGGEEDITVQTVTWPDMELPLPRNITEGEARGSVILTVKPIFEVSPSPLEPEEPFTFAPEIGATAFAEVENETGEATRPWGFPTPGLGPATAFTSEDLVVQVTAVPGQPHLPGGVVFHYRPGPTRYSLTFEEAQQACPGTGAVIASPEQLQAAYEAGYEQCDAGWLRDQTVRYPIVSPRTPCVGDKDSSPGVRTYGVRPSTETYDVYCFVDRLEGEVFFATRLEQFTFQEALEFCESHNATATTGQLYAAWSRGLDKCYAGWLADGSLRYPIVTPRPACGGDKPGVRTVYLYPNQTGLPDPLSRHHAFCFRGISAVPSPGEEEGGTPTSPSGVEEWIVTQVVPGVAAVPVEEETTAVPSGETTAILEFTTEPENQTEWEPAYTPVGTSPLPGILPTWPPTGAETEESTEGPSATEVPSASEEPSPSEVPFPSEEPSPSEEPFPSVRPFPSVELFPSEEPFPSKEPSPSEEPSASEEPYTPSPPEPSWTELPSSGEESGAPDVSGDFTGSGDVSGHLDFSGQLSGDRASGLPSGDLDSSGLTSTVGSGLTVESGLPSGDEERIEWPSTPTVGELPSGAEILEGSASGVGDLSGLPSGEVLETSASGVGDLSGLPSGEVLETTAPGVEDISGLPSGEVLETTAPGVEDISGLPSGEVLETTAPGVEDISGLPSGEVLETTAPGVEDISGLPSGEVLETTAPGVEDISGLPSGEVLETAAPGVEDISGLPSGEVLETAAPGVEDISGLPSGEVLETAAPGVEDISGLPSGEVLETAAPGVEDISGLPSGEVLETAAPGVEDISGLPSGEVLETAAPGVEDISGLPSGEVLETAAPGVEDISGLPSGEVLETAAPGVEDISGLPSGEVLETAAPGVEDISGLPSGEVLETAAPGVEDISGLPSGEVLETAAPGVEDISGLPSGEVLETTAPGVEEISGLPSGEVLETTAPGVDEISGLPSGEVLETTAPGVEEISGLPSGEVLETSTSAVGDLSGLPSGGEVLEISVSGVEDISGLPSGEVVETSASGIEDVSELPSGEGLETSASGVEDLSRLPSGEEVLEISASGFGDLSGVPSGGEGLETSASEVGTDLSGLPSGREGLETSASGAEDLSGLPSGKEDLVGSASGDLDLGKLPSGTLGSGQAPETSGLPSGFSGEYSGVDLGSGPPSGLPDFSGLPSGFPTVSLVDSTLVEVVTASTASELEGRGTIGISGAGEISGLPSSELDISGRASGLPSGTELSGQASGSPDVSGEIPGLFGVSGQPSGFPDTSGETSGVTELSGLSSGQPGVSGEASGVLYGTSQPFGITDLSGETSGVPDLSGQPSGLPGFSGATSGVPDLVSGTTSGSGESSGITFVDTSLVEVAPTTFKEEEGLGSVELSGLPSGEADLSGKSGMVDVSGQFSGTVDSSGFTSQTPEFSGLPSGIAEVSGESSRAEIGSSLPSGAYYGSGTPSSFPTVSLVDRTLVESVTQAPTAQEAGEGPSGILELSGAHSGAPDMSGEHSGFLDLSGLQSGLIEPSGEPPGTPYFSGDFASTTNVSGESSVAMGTSGEASGLPEVTLITSEFVEGVTEPTISQELGQRPPVTHTPQLFESSGKVSTAGDISGATPVLPGSGVEVSSVPESSSETSAYPEAGFGASAAPEASREDSGSPDLSETTSAFHEANLERSSGLGVSGSTLTFQEGEASAAPEVSGESTTTSDVGTEAPGLPSATPTASGDRTEISGDLSGHTSQLGVVISTSIPESEWTQQTQRPAETHLEIESSSLLYSGEETHTVETATSPTDASIPASPEWKRESESTAAAPARSCAEEPCGAGTCKETEGHVICLCPPGYTGEHCNIDQEVCEEGWNKYQGHCYRHFPDRETWVDAERRCREQQSHLSSIVTPEEQEFVNNNAQDYQWIGLNDRTIEGDFRWSDGHPMQFENWRPNQPDNFFAAGEDCVVMIWHEKGEWNDVPCNYHLPFTCKKGTVACGEPPVVEHARTFGQKKDRYEINSLVRYQCTEGFVQRHMPTIRCQPSGHWEEPRITCTDATTYKRRLQKRSSRHPRRSRPSTAH

SEQ ID NO: 156 - protein, 122 aa, synthetic construct
  REGION 1..122: note = Amino acid sequence
EVQLVESGGGVVQPGGSLRLSCAASGSTFIINVVRWYRRAPGKQRELVATISSGGNANYVDSVRGRFTISRDNSKNTVYLQMNSLRPEDTALYYCNVPTTHYGGVYYGPYWGQGTLVTVSSA

SEQ ID NO: 157 - protein, 125 aa, synthetic construct
  REGION 1..125: note = Amino acid sequence
EVQLVESGGGVVQPGGSLRLSCAASGRTFSSYTMGWFRQAPGKEREFVAAISWSGGRTYYADSVKGRFTISRDNSKNTVYLQMNSLRPEDTALYYCAAYRRRRASSNRGLWDYWGQGTLVTVSSA

SEQ ID NO: 158 - skipped

SEQ ID NO: 159 - protein, 5 aa, synthetic construct
  REGION 1..5: note = Amino acid sequence
GGGGS

SEQ ID NO: 160 - protein, 7 aa, synthetic construct
  REGION 1..7: note = Amino acid sequence
SGGSGGS

SEQ ID NO: 161 - protein, 8 aa, synthetic construct
  REGION 1..8: note = Amino acid sequence
GGGGGGGS

SEQ ID NO: 162 - protein, 9 aa, synthetic construct
  REGION 1..9: note = Amino acid sequence
GGGGSGGGS

SEQ ID NO: 163 - protein, 10 aa, synthetic construct
  REGION 1..10: note = Amino acid sequence
GGGGSGGGGS

SEQ ID NO: 164 - protein, 15 aa, synthetic construct
  REGION 1..15: note = Amino acid sequence
GGGGSGGGGSGGGGS

SEQ ID NO: 165 - protein, 18 aa, synthetic construct
  REGION 1..18: note = Amino acid sequence
GGGGSGGGGSGGGGGGGS

SEQ ID NO: 166 - protein, 20 aa, synthetic construct
  REGION 1..20: note = Amino acid sequence
GGGGSGGGGSGGGGSGGGGS

SEQ ID NO: 167 - protein, 25 aa, synthetic construct
  REGION 1..25: note = Amino acid sequence
GGGGSGGGGSGGGGSGGGGSGGGGS

SEQ ID NO: 168 - protein, 30 aa, synthetic construct
  REGION 1..30: note = Amino acid sequence
GGGGSGGGGSGGGGSGGGGSGGGGSGGGGS

SEQ ID NO: 169 - protein, 35 aa, synthetic construct
  REGION 1..35: note = Amino acid sequence
GGGGSGGGGSGGGGSGGGGSGGGGSGGGGSGGGGS

SEQ ID NO: 170 - protein, 40 aa, synthetic construct
  REGION 1..40: note = Amino acid sequence
GGGGSGGGGSGGGGSGGGGSGGGGSGGGGSGGGGSGGGGS

SEQ ID NO: 171 - protein, 15 aa, synthetic construct
  REGION 1..15: note = Amino acid sequence
EPKSCDKTHTCPPCP

SEQ ID NO: 172 - protein, 24 aa, synthetic construct
  REGION 1..24: note = Amino acid sequence
GGGGSGGGSEPKSCDKTHTCPPCP

SEQ ID NO: 173 - protein, 12 aa, synthetic construct
  REGION 1..12: note = Amino acid sequence
EPKTPKPQPAAA

SEQ ID NO: 174 - protein, 62 aa, synthetic construct
  REGION 1..62: note = Amino acid sequence
ELKTPLGDTTHTCPRCPEPKSCDTPPPCPRCPEPKSCDTPPPCPRCPEPKSCDTPPPCPRCP